European Patent Specification EP 3 866 826 B1, published December 10, 2025. Title: ANTIMICROBIAL PEPTIDES AND METHODS OF USING THE SAME. Applicant: Riptide Bioscience, Inc. The sequence listing filed with the application follows.

SEQUENCE LISTING (81 sequences)

SEQ ID NO: 1 - protein, 19 aa, Artificial Sequence
  Synthetic sequence
  misc_feature (4)..(4): Xaa is ornithine
  misc_feature (11)..(11): Xaa is ornithine
  misc_feature (15)..(15): Xaa is ornithine
FKIXARLCLGXFCIXARLK

SEQ ID NO: 2 - protein, 23 aa, Artificial Sequence
  Synthetic sequence
  misc_feature (3)..(3): Xaa is ornithine
  misc_feature (8)..(8): Xaa is ornithine
  misc_feature (11)..(11): Xaa is ornithine
  misc_feature (14)..(14): Xaa is ornithine
FIXKFAKXFKXFIXKFAKFAFAF

SEQ ID NO: 3 - protein, 23 aa, Artificial Sequence
  Synthetic sequence
  misc_feature (14)..(14): Xaa is ornithine
  misc_feature (16)..(17): Xaa is ornithine
  misc_feature (20)..(21): Xaa is ornithine
FAFAFKAFKKAFKXFXXAFXXAF

SEQ ID NO: 4 - protein, 17 aa, Artificial Sequence
  Synthetic sequence
  misc_feature (2)..(2): Xaa is ornithine
  misc_feature (8)..(8): Xaa is ornithine
  misc_feature (14)..(14): Xaa is ornithine
FXIKARFXVRARLXLKI

SEQ ID NO: 5 - protein, 17 aa, Artificial Sequence
  Synthetic sequence
FRLKIKARLKVKIRFKL

SEQ ID NO: 6 - protein, 17 aa, Artificial Sequence
  Synthetic sequence
  misc_feature (2)..(2): Xaa is ornithine
  misc_feature (4)..(4): Xaa is ornithine
  misc_feature (6)..(6): Xaa is ornithine
  misc_feature (8)..(8): Xaa is ornithine
  misc_feature (10)..(10): Xaa is ornithine
  misc_feature (12)..(12): Xaa is ornithine
  misc_feature (14)..(14): Xaa is ornithine
  misc_feature (16)..(16): Xaa is ornithine
FXLXAXIXVXLXAXIXL

SEQ ID NO: 7 - protein, 17 aa, Artificial Sequence
  Synthetic sequence
  misc_feature (2)..(2): Xaa is ornithine
  misc_feature (4)..(4): Xaa is ornithine
  misc_feature (6)..(6): Xaa is ornithine
  misc_feature (12)..(12): Xaa is ornithine
  misc_feature (14)..(14): Xaa is ornithine
  misc_feature (16)..(16): Xaa is ornithine
FXLXAXIKVKLXAXIXL

SEQ ID NO: 8 - protein, 17 aa, Artificial Sequence
  Synthetic sequence
RFCWKVCYKGICFKKCK

SEQ ID NO: 9 - protein, 17 aa, Artificial Sequence
  Synthetic sequence
RCRRYCIGRYCVRFCWK

SEQ ID NO: 10 - protein, 17 aa, Artificial Sequence
  Synthetic sequence
  misc_feature (1)..(1): Xaa is ornithine
  misc_feature (5)..(5): Xaa is ornithine
  misc_feature (9)..(9): Xaa is ornithine
  misc_feature (14)..(15): Xaa is ornithine
  misc_feature (17)..(17): Xaa is ornithine
XWCFXVCYXGICYXXCX

SEQ ID NO: 11 - protein, 17 aa, Artificial Sequence
  Synthetic sequence
RWCFKVCYKGICYKKCK

SEQ ID NO: 12 - protein, 17 aa, Artificial Sequence
  Synthetic sequence
  misc_feature (1)..(1): Xaa is ornithine
  misc_feature (5)..(5): Xaa is ornithine
  misc_feature (9)..(9): Xaa is ornithine
  misc_feature (14)..(15): Xaa is ornithine
  misc_feature (17)..(17): Xaa is ornithine
XFCWXVCYXGICFXXCX

SEQ ID NO: 13 - protein, 17 aa, Artificial Sequence
  Synthetic sequence
  misc_feature (1)..(1): Xaa is ornithine
  misc_feature (3)..(4): Xaa is ornithine
  misc_feature (9)..(9): Xaa is ornithine
  misc_feature (13)..(13): Xaa is ornithine
  misc_feature (17)..(17): Xaa is ornithine
XCXXFCIGXYCVXWCFX

SEQ ID NO: 14 - protein, 18 aa, Artificial Sequence
  Synthetic sequence
RGVCVCFRRRCYCLRGGR

SEQ ID NO: 15 - protein, 24 aa, Artificial Sequence
  Synthetic sequence
  misc_feature (2)..(2): Xaa is ornithine
  misc_feature (4)..(4): Xaa is ornithine
  misc_feature (6)..(6): Xaa is ornithine
  misc_feature (13)..(13): Xaa is ornithine
  misc_feature (19)..(19): Xaa is ornithine
  misc_feature (21)..(21): Xaa is ornithine
  misc_feature (23)..(23): Xaa is ornithine
FXIXAXLGGCLGXFCGGIXAXLXF

SEQ ID NO: 16 - protein, 26 aa, Artificial Sequence
  Synthetic sequence
  misc_feature (2)..(2): Xaa is ornithine
  misc_feature (4)..(4): Xaa is ornithine
  misc_feature (6)..(6): Xaa is ornithine
  misc_feature (8)..(8): Xaa is ornithine
  misc_feature (14)..(14): Xaa is ornithine
  misc_feature (19)..(19): Xaa is ornithine
  misc_feature (21)..(21): Xaa is ornithine
  misc_feature (23)..(23): Xaa is ornithine
  misc_feature (25)..(25): Xaa is ornithine
FXIXAXLXGGCLGXFCGGXIXAXLXF

SEQ ID NO: 17 - protein, 24 aa, Artificial Sequence
  Synthetic sequence
  misc_feature (2)..(2): Xaa is ornithine
  misc_feature (6)..(6): Xaa is ornithine
  misc_feature (21)..(21): Xaa is ornithine
FXIKAXLGGCLGKFCGGIKAXLKF

SEQ ID NO: 18 - protein, 26 aa, Artificial Sequence
  Synthetic sequence
  misc_feature (2)..(2): Xaa is ornithine
  misc_feature (6)..(6): Xaa is ornithine
  misc_feature (23)..(23): Xaa is ornithine
FXIKAXLKGGCLGKFCGGKIKAXLKF

SEQ ID NO: 19 - protein, 5 aa, Artificial Sequence
  Synthetic sequence
FAFAF

SEQ ID NO: 20 - protein, 5 aa, Artificial Sequence
  Synthetic sequence
AFAFA

SEQ ID NO: 21 - protein, 6 aa, Artificial Sequence
  Synthetic sequence
CLGRFC

SEQ ID NO: 22 - protein, 6 aa, Artificial Sequence
  Synthetic sequence
CYKGIC

SEQ ID NO: 23 - protein, 6 aa, Artificial Sequence
  Synthetic sequence
  misc_feature (1)..(1): Xaa is a hydrophobic amino acid residue or a hydrophilic amino acid residue
  misc_feature (6)..(6): Xaa is a hydrophobic amino acid residue or a hydrophilic amino acid residue
XGPGRX

SEQ ID NO: 24 - protein, 17 aa, Artificial Sequence
  Synthetic sequence
  misc_feature (2)..(2): Xaa is Ornithine
  misc_feature (3)..(3): Xaa is I or L
  misc_feature (4)..(4): Xaa is ornithine or K
  misc_feature (6)..(6): Xaa is ornithine or R
  misc_feature (7)..(7): Xaa is I or F
  misc_feature (8)..(8): Xaa is ornithine or K
  misc_feature (10)..(10): Xaa is Ornithine, K, or R
  misc_feature (11)..(11): Xaa is A or L
  misc_feature (12)..(12): Xaa is ornithine or R
  misc_feature (13)..(13): Xaa is A or L
  misc_feature (14)..(14): Xaa is ornithine
  misc_feature (15)..(15): Xaa is I or L
  misc_feature (16)..(16): Xaa is ornithine or K
  misc_feature (17)..(17): Xaa is I or L
FXXXAXXXVXXXXXXXX

SEQ ID NO: 25 - protein, 11 aa, Artificial Sequence
  Synthetic sequence
  misc_feature (4)..(4): Xaa is a hydrophobic amino acid residue or a hydrophilic amino acid residue
  misc_feature (5)..(5): Xaa is a hydrophobic amino acid residue or a hydrophilic amino acid residue
  misc_feature (6)..(6): Xaa is a hydrophobic amino acid residue or a hydrophilic amino acid residue
  misc_feature (7)..(7): Xaa is a hydrophobic amino acid residue, a hydrophilic amino acid residue, or is not present
  misc_feature (8)..(8): Xaa is a hydrophobic amino acid residue, a hydrophilic amino acid residue, or is not present
GGCXXXXXCGG

SEQ ID NO: 26 - protein, 8 aa, Artificial Sequence
  Synthetic sequence
  misc_feature (1)..(1): This stretch of residues may be repeated
  misc_feature (3)..(3): Xaa is a hydrophobic amino acid residue
  misc_feature (4)..(4): Xaa is a hydrophobic amino acid residue
  misc_feature (5)..(5): Xaa is a hydrophilic amino acid residue
  misc_feature (6)..(6): Xaa is a hydrophobic amino acid residue
  misc_feature (8)..(8): This stretch of residues may be repeated
GCXXXXCG

SEQ ID NO: 27 - protein, 17 aa, Artificial Sequence
  Synthetic sequence
  misc_feature (2)..(2): Xaa is ornithine or K
  misc_feature (4)..(4): Xaa is ornithine or K
  misc_feature (6)..(6): Xaa is ornithine or R
  misc_feature (8)..(8): Xaa is ornithine or K
  misc_feature (9)..(9): Xaa is a naturally occuring amino acid
  misc_feature (10)..(10): Xaa is ornithine or K
  misc_feature (12)..(12): Xaa is ornithine or K
  misc_feature (14)..(14): Xaa is ornithine or R
  misc_feature (16)..(16): Xaa is ornithine or K
FXIXAXLXXXIXAXLXF

SEQ ID NO: 28 - protein, 6 aa, Artificial Sequence
  Synthetic sequence
  misc_feature (4)..(4): Xaa is Ornithine or K
CLGXFC

SEQ ID NO: 29 - protein, 8 aa, Artificial Sequence
  Synthetic sequence
  misc_feature (5)..(5): Xaa is Ornithine or K
GCLGXFCG

SEQ ID NO: 30 - protein, 10 aa, Artificial Sequence
  Synthetic sequence
  misc_feature (6)..(6): Xaa is Ornithine or K
GGCLGXFCGG

SEQ ID NO: 31 - protein, 24 aa, Artificial Sequence
  Synthetic sequence
  misc_feature (1)..(1): Xaa is a hydrophobic amino acid residue
  misc_feature (2)..(2): Xaa is a hydrophilic amino acid residue
  misc_feature (3)..(3): Xaa is a hydrophobic amino acid residue
  misc_feature (4)..(4): Xaa is a hydrophilic amino acid residue
  misc_feature (5)..(5): Xaa is a hydrophobic amino acid residue
  misc_feature (6)..(6): Xaa is a hydrophilic amino acid residue
  misc_feature (7)..(7): Xaa is a hydrophobic amino acid residue
  misc_feature (11)..(11): Xaa is a hydrophobic amino acid residue
  misc_feature (12)..(12): Xaa is a hydrophobic amino acid residue
  misc_feature (13)..(13): Xaa is a hydrophilic amino acid residue
  misc_feature (14)..(14): Xaa is a hydrophobic amino acid residue
  misc_feature (18)..(18): Xaa is a hydrophobic amino acid residue
  misc_feature (19)..(19): Xaa is a hydrophilic amino acid residue
  misc_feature (20)..(20): Xaa is a hydrophobic amino acid residue
  misc_feature (21)..(21): Xaa is a hydrophilic amino acid residue
  misc_feature (22)..(22): Xaa is a hydrophobic amino acid residue
  misc_feature (23)..(23): Xaa is a a hydrophilic amino acid residue
  misc_feature (24)..(24): Xaa is a hydrophobic amino acid residue
XXXXXXXGGCXXXXCGGXXXXXXX

SEQ ID NO: 32 - protein, 26 aa, Artificial Sequence
  Synthetic sequence
  misc_feature (1)..(1): Xaa is a hydrophobic amino acid residue
  misc_feature (2)..(2): Xaa is a hydrophilic amino acid residue
  misc_feature (3)..(3): Xaa is a hydrophobic amino acid residue
  misc_feature (4)..(4): Xaa is a hydrophilic amino acid residue
  misc_feature (5)..(5): Xaa is a hydrophobic amino acid residue
  misc_feature (6)..(6): Xaa is a hydrophilic amino acid residue
  misc_feature (7)..(7): Xaa is a hydrophobic amino acid residue
  misc_feature (8)..(8): Xaa is a hydrophilic amino acid residue
  misc_feature (12)..(12): Xaa is a hydrophobic amino acid residue
  misc_feature (13)..(13): Xaa is a hydrophobic amino acid residue
  misc_feature (14)..(14): Xaa is a hydrophilic amino acid residue
  misc_feature (15)..(15): Xaa is a hydrophobic amino acid residue
  misc_feature (19)..(19): Xaa is a hydrophilic amino acid residue
  misc_feature (20)..(20): Xaa is a hydrophobic amino acid residue
  misc_feature (21)..(21): Xaa is a hydrophilic amino acid residue
  misc_feature (22)..(22): Xaa is a hydrophobic amino acid residue
  misc_feature (23)..(23): Xaa is a hydrophilic amino acid residue
  misc_feature (24)..(24): Xaa is a hydrophobic amino acid residue
  misc_feature (25)..(25): Xaa is a hydrophilic amino acid residue
  misc_feature (26)..(26): Xaa is a hydrophobic amino acid residue
XXXXXXXXGGCXXXXCGGXXXXXXXX

SEQ ID NO: 33 - protein, 7 aa, Artificial Sequence
  Synthetic sequence
  misc_feature (2)..(2): Xaa is Ornithine or K
  misc_feature (4)..(4): Xaa is Ornithine or K
  misc_feature (6)..(6): Xaa is Ornithine or R
FXIXAXL

SEQ ID NO: 34 - protein, 7 aa, Artificial Sequence
  Synthetic sequence
  misc_feature (4)..(4): Xaa is Ornithine
FKIXARL

SEQ ID NO: 35 - protein, 7 aa, Artificial Sequence
  Synthetic sequence
  misc_feature (2)..(2): Xaa is Ornithine
  misc_feature (4)..(4): Xaa is Ornithine
  misc_feature (6)..(6): Xaa is Ornithine
FXIXAXL

SEQ ID NO: 36 - protein, 7 aa, Artificial Sequence
  Synthetic sequence
  misc_feature (2)..(2): Xaa is Ornithine
  misc_feature (6)..(6): Xaa is Ornithine
FXIKAXL

SEQ ID NO: 37 - protein, 7 aa, Artificial Sequence
  Synthetic sequence
  misc_feature (2)..(2): Xaa is Ornithine or K
  misc_feature (4)..(4): Xaa is Ornithine or R
  misc_feature (6)..(6): Xaa is Ornithine or K
IXAXLXF

SEQ ID NO: 38 - protein, 6 aa, Artificial Sequence
  Synthetic sequence
  misc_feature (2)..(2): Xaa is Ornithine
IXARLK

SEQ ID NO: 39 - protein, 7 aa, Artificial Sequence
  Synthetic sequence
  misc_feature (2)..(2): Xaa is Ornithine
  misc_feature (4)..(4): Xaa is Ornithine
  misc_feature (6)..(6): Xaa is Ornithine
IXAXLXF

SEQ ID NO: 40 - protein, 7 aa, Artificial Sequence
  Synthetic sequence
  misc_feature (4)..(4): Xaa is Ornithine
IKAXLKF

SEQ ID NO: 41 - protein, 6 aa, Artificial Sequence
  Synthetic sequence
  misc_feature (4)..(4): Xaa is Ornithine
CLGXFC

SEQ ID NO: 42 - protein, 6 aa, Artificial Sequence
  Synthetic sequence
CLGKFC

SEQ ID NO: 43 - protein, 8 aa, Artificial Sequence
  Synthetic sequence
  misc_feature (6)..(6): Xaa is Ornithine
GGCLGXFC

SEQ ID NO: 44 - protein, 10 aa, Artificial Sequence
  Synthetic sequence
GGCLGKFCGG

SEQ ID NO: 45 - protein, 9 aa, Artificial Sequence
  Synthetic sequence
  misc_feature (1)..(1): Xaa is a naturally occuring amino acid
  misc_feature (3)..(3): Xaa is a naturally occuring amino acid
  misc_feature (5)..(5): Xaa is a naturally occuring amino acid
  misc_feature (7)..(7): Xaa is a naturally occuring amino acid
  misc_feature (9)..(9): Xaa is a naturally occuring amino acid
XCXCXCXCX

SEQ ID NO: 46 - protein, 17 aa, Artificial Sequence
  Synthetic sequence
  misc_feature (1)..(1): Xaa  is a hydrophilic amino acid residue
  misc_feature (2)..(2): Xaa  is a hydrophobic amino acid residue
  misc_feature (4)..(4): Xaa  is a hydrophobic amino acid residue
  misc_feature (5)..(5): Xaa  is a hydrophilic amino acid residue
  misc_feature (6)..(6): Xaa is a hydrophobic amino acid residue
  misc_feature (8)..(8): Xaa  is a hydrophobic amino acid residue
  misc_feature (9)..(9): Xaa  is a hydrophilic amino acid residue
  misc_feature (10)..(10): Xaa is a hydrophobic amino acid residue
  misc_feature (11)..(11): Xaa is a hydrophobic amino acid residue
  misc_feature (13)..(13): Xaa is a hydrophobic amino acid residue
  misc_feature (14)..(14): Xaa is a hydrophilic amino acid residue
  misc_feature (15)..(15): Xaa is a hydrophilic amino acid residue
  misc_feature (17)..(17): Xaa is a hydrophilic amino acid residue
XXCXXXCXXXXCXXXCX

SEQ ID NO: 47 - protein, 17 aa, Artificial Sequence
  Synthetic sequence
  misc_feature (1)..(1): Xaa is Ornithine or R
  misc_feature (2)..(2): Xaa is F or W
  misc_feature (4)..(4): Xaa is F or W
  misc_feature (5)..(5): Xaa is Ornithine or K
  misc_feature (9)..(9): Xaa is Ornithine or K
  misc_feature (13)..(13): Xaa is F or W
  misc_feature (14)..(14): Xaa is Ornithine or K
  misc_feature (15)..(15): Xaa is Ornithine or K
  misc_feature (17)..(17): Xaa is Ornithine or K
XXCXXVCYXGICXXXCX

SEQ ID NO: 48 - protein, 17 aa, Artificial Sequence
  Synthetic sequence
  misc_feature (1)..(1): Xaa is a hydrophilic amino acid residue
  misc_feature (3)..(3): Xaa is a hydrophilic amino acid residue
  misc_feature (4)..(4): Xaa is a hydrophilic amino acid residue
  misc_feature (5)..(5): Xaa is a hydrophobic amino acid residue
  misc_feature (7)..(7): Xaa is a hydrophobic amino acid residue
  misc_feature (8)..(8): Xaa is a hydrophobic amino acid residue
  misc_feature (9)..(9): Xaa is a hydrophilic amino acid residue
  misc_feature (10)..(10): Xaa is a hydrophobic amino acid residue
  misc_feature (12)..(12): Xaa is a hydrophobic amino acid residue
  misc_feature (13)..(13): Xaa is a hydrophilic amino acid residue
  misc_feature (14)..(14): Xaa is a hydrophobic amino acid residue
  misc_feature (16)..(16): Xaa is a hydrophobic amino acid residue
  misc_feature (17)..(17): Xaa is a hydrophilic amino acid residue
XCXXXCXXXXCXXXCXX

SEQ ID NO: 49 - protein, 17 aa, Artificial Sequence
  Synthetic sequence
  misc_feature (1)..(1): Xaa is a Ornithine or R
  misc_feature (3)..(3): Xaa is a Ornithine or R
  misc_feature (4)..(4): Xaa is a Ornithine or R
  misc_feature (5)..(5): Xaa is Y or F
  misc_feature (9)..(9): Xaa is a Ornithine or R
  misc_feature (13)..(13): Xaa is a Ornithine or R
  misc_feature (14)..(14): Xaa is F or W
  misc_feature (16)..(16): Xaa is F or W
  misc_feature (17)..(17): Xaa is Ornithine or K
XCXXXCIGXYCVXXCXX

SEQ ID NO: 50 - protein, 18 aa, Artificial Sequence
  Synthetic sequence
  misc_feature (1)..(1): Xaa is a hydrophilic amino acid residue
  misc_feature (2)..(2): Xaa is a hydrophobic amino acid residue
  misc_feature (3)..(3): Xaa is a hydrophobic amino acid residue
  misc_feature (5)..(5): Xaa is a hydrophobic amino acid residue
  misc_feature (7)..(7): Xaa is a hydrophobic amino acid residue
  misc_feature (8)..(8): Xaa is a hydrophilic amino acid residue
  misc_feature (9)..(9): Xaa is a hydrophilic amino acid residue
  misc_feature (10)..(10): Xaa is a hydrophilic amino acid residue
  misc_feature (12)..(12): Xaa is a hydrophobic amino acid residue
  misc_feature (14)..(14): Xaa is a hydrophobic amino acid residue
  misc_feature (15)..(15): Xaa is a hydrophilic amino acid residue
  misc_feature (16)..(16): Xaa is a hydrophobic amino acid residue
  misc_feature (17)..(17): Xaa is a hydrophobic amino acid residue
  misc_feature (18)..(18): Xaa is a hydrophilic amino acid residue
XXXCXCXXXXCXCXXXXX

SEQ ID NO: 51 - protein, 6 aa, Artificial Sequence
  Synthetic sequence
  misc_feature (3)..(3): Xaa is Ornithine
CYXGIC

SEQ ID NO: 52 - protein, 6 aa, Artificial Sequence
  Synthetic sequence
CIGRYC

SEQ ID NO: 53 - protein, 6 aa, Artificial Sequence
  Synthetic sequence
  misc_feature (4)..(4): Xaa is Ornithine
CIGXYC

SEQ ID NO: 54 - protein, 6 aa, Artificial Sequence
  Synthetic sequence
CFRRRC

SEQ ID NO: 55 - protein, 18 aa, Artificial Sequence
  Synthetic sequence
  misc_feature (3)..(3): Xaa is Ornithine
  misc_feature (8)..(8): Xaa is Ornithine
  misc_feature (11)..(11): Xaa is Ornithine
  misc_feature (14)..(14): Xaa is Ornithine
FIXKFAKXFKXFIXKFAK

SEQ ID NO: 56 - protein, 18 aa, Artificial Sequence
  Synthetic sequence
RVFKKAFRKFKKLFKRAF

SEQ ID NO: 57 - protein, 18 aa, Artificial Sequence
  Synthetic sequence
FARKFLKKFKRFAKKFVR

SEQ ID NO: 58 - protein, 18 aa, Artificial Sequence
  Synthetic sequence
FKRKIKAKLRFKAKVRLK

SEQ ID NO: 59 - protein, 23 aa, Artificial Sequence
  Synthetic sequence
FAFAFRVFKKAFRKFKKLFKRAF

SEQ ID NO: 60 - protein, 23 aa, Artificial Sequence
  Synthetic sequence
FARKFLKKFKRFAKKFVRFAFAF

SEQ ID NO: 61 - protein, 18 aa, Artificial Sequence
  Synthetic sequence
KIRAKLCLGRFCIRAKLR

SEQ ID NO: 62 - protein, 18 aa, Artificial Sequence
  Synthetic sequence
KIKARLCLGKFCIKARLK

SEQ ID NO: 63 - protein, 50 aa, Artificial Sequence
  Synthetic sequence
FAFAFKAFKKAFKKFKKAFKKAFGPGRFAKKFAKKFKKFAKKFAKFAFAF

SEQ ID NO: 64 - protein, 50 aa, Artificial Sequence
  Synthetic sequence
FAKKFAKKFKKFAKKFAKFAFAFGPGRFAFAFKAFKKAFKKFKKAFKKAF

SEQ ID NO: 65 - protein, 19 aa, Artificial Sequence
  Synthetic sequence
MGFKLRAKIKVRLRAKIKL

SEQ ID NO: 66 - protein, 12 aa, Artificial Sequence
  Synthetic sequence
  misc_feature (3)..(3): Xaa is Ornithine
  misc_feature (8)..(8): Xaa is Ornithine
CVXLFPVXLFPC

SEQ ID NO: 67 - protein, 16 aa, Artificial Sequence
  Synthetic sequence
CKLRFRGPGRIKVRLC

SEQ ID NO: 68 - protein, 26 aa, Artificial Sequence
  Synthetic sequence
CPGFAKKFAKKFKKFAKKFAKFAFAF

SEQ ID NO: 69 - protein, 18 aa, Artificial Sequence
  Synthetic sequence
KIRAKLCLGRFCIRAKLR

SEQ ID NO: 70 - protein, 26 aa, Artificial Sequence
  Synthetic sequence
KKKPKPPYLPKPKPPPFFPPKLPPKI

SEQ ID NO: 71 - protein, 26 aa, Artificial Sequence
  Synthetic sequence
FAFAFKAFKKAFKKFKKAFKKAFGPC

SEQ ID NO: 72 - protein, 22 aa, Artificial Sequence
  Synthetic sequence
FAFAFAFKKAFKKFKKAFKKAF

SEQ ID NO: 73 - protein, 23 aa, Artificial Sequence
  Synthetic sequence
  misc_feature (6)..(6): Xaa is Ornithine
  misc_feature (9)..(10): Xaa is Ornithine
  misc_feature (13)..(13): Xaa is Ornithine
  misc_feature (14)..(14): Xaa is Ornithine
  misc_feature (16)..(16): Xaa is Ornithine
  misc_feature (17)..(17): Xaa is Ornithine
  misc_feature (20)..(20): Xaa is Ornithine
  misc_feature (21)..(21): Xaa is Ornithine
FAFAFXAFXXAFXXFXXAFXXAF

SEQ ID NO: 74 - protein, 23 aa, Artificial Sequence
  Synthetic sequence
  misc_feature (3)..(3): Xaa is Ornithine
  misc_feature (4)..(4): Xaa is Ornithine
  misc_feature (7)..(7): Xaa is Ornithine
  misc_feature (8)..(8): Xaa is Ornithine
  misc_feature (10)..(10): Xaa is Ornithine
  misc_feature (11)..(11): Xaa is Ornithine
  misc_feature (14)..(14): Xaa is Ornithine
  misc_feature (15)..(15): Xaa is Ornithine
  misc_feature (18)..(18): Xaa is Ornithine
FAXXFAXXFXXFAXXFAXFAFAF

SEQ ID NO: 75 - protein, 22 aa, Artificial Sequence
  Synthetic sequence
FAKKFAKKFKKFAKKFAFAFAF

SEQ ID NO: 76 - protein, 31 aa, Artificial Sequence
  Synthetic sequence
  misc_feature (11)..(11): Xaa is Ornithine
  misc_feature (12)..(12): Xaa is Ornithine
  misc_feature (15)..(15): Xaa is Ornithine
  misc_feature (16)..(16): Xaa is Ornithine
  misc_feature (18)..(18): Xaa is Ornithine
  misc_feature (19)..(19): Xaa is Ornithine
  misc_feature (22)..(22): Xaa is Ornithine
  misc_feature (23)..(23): Xaa is Ornithine
  misc_feature (26)..(26): Xaa is Ornithine
RLARIVGGFAXXFAXXFXXFAXXFAXFAFAF

SEQ ID NO: 77 - protein, 33 aa, Artificial Sequence
  Synthetic sequence
  misc_feature (13)..(13): Xaa is Ornithine
  misc_feature (14)..(14): Xaa is Ornithine
  misc_feature (17)..(17): Xaa is Ornithine
  misc_feature (18)..(18): Xaa is Ornithine
  misc_feature (20)..(20): Xaa is Ornithine
  misc_feature (21)..(21): Xaa is Ornithine
  misc_feature (24)..(24): Xaa is Ornithine
  misc_feature (25)..(25): Xaa is Ornithine
  misc_feature (28)..(28): Xaa is Ornithine
CRLARIVCGGFAXXFAXXFXXFAXXFAXFAFAF

SEQ ID NO: 78 - protein, 24 aa, Artificial Sequence
  Synthetic sequence
  misc_feature (2)..(2): Xaa is Ornithine
  misc_feature (4)..(4): Xaa is Ornithine
  misc_feature (6)..(6): Xaa is Ornithine
  misc_feature (13)..(13): Xaa is Ornithine
  misc_feature (19)..(19): Xaa is Ornithine
  misc_feature (21)..(21): Xaa is Ornithine
  misc_feature (23)..(23): Xaa is Ornithine
FXIXAXLGGCLGXFCGGIXAXLXF

SEQ ID NO: 79 - protein, 26 aa, Artificial Sequence
  Synthetic sequence
  misc_feature (1)..(1): Xaa is Ornithine
  misc_feature (3)..(3): Xaa is Ornithine
  misc_feature (11)..(11): Xaa is Ornithine
  misc_feature (13)..(13): Xaa is Ornithine
  misc_feature (14)..(14): Xaa is Ornithine
  misc_feature (15)..(15): Xaa is Ornithine
  misc_feature (16)..(16): Xaa is Ornithine
  misc_feature (18)..(18): Xaa is Ornithine
  misc_feature (20)..(20): Xaa is Ornithine
  misc_feature (21)..(21): Xaa is Ornithine
  misc_feature (22)..(22): Xaa is Ornithine
  misc_feature (26)..(26): Xaa is Ornithine
XLXSLLKTLSXAXXXXLXTXXXAISX

SEQ ID NO: 80 - protein, 27 aa, Artificial Sequence
  Synthetic sequence
  misc_feature (7)..(7): Xaa is Ornithine
  misc_feature (8)..(8): Xaa is Ornithine
  misc_feature (9)..(9): Xaa is Ornithine
  misc_feature (12)..(12): Xaa is Ornithine
  misc_feature (14)..(14): Xaa is Ornithine
  misc_feature (16)..(16): Xaa is Ornithine
ALWMTLXXXVLXAXAXALNAVLVGANA

SEQ ID NO: 81 - protein, 27 aa, Artificial Sequence
  Synthetic sequence
  misc_feature (7)..(7): Xaa is Ornithine
  misc_feature (8)..(8): Xaa is Ornithine
  misc_feature (9)..(9): Xaa is Ornithine
  misc_feature (12)..(12): Xaa is Ornithine
  misc_feature (14)..(14): Xaa is Ornithine
  misc_feature (16)..(16): Xaa is Ornithine
AFAFTAXXXFAXFXAXFANFAFAGFNA